European Patent Specification EP 3 768 701 B1, published August 2, 2023. Title: WNT SIGNALING AGONIST MOLECULES. Applicant: Université Libre de Bruxelles. The sequence listing filed with the application follows.

SEQUENCE LISTING (121 sequences)

SEQ ID NO: 1 - protein, 1338 aa, homo sapiens
MGAGGRRMRGAPARLLLPLLPWLLLLLAPEARGAPGCPLSIRSCKCSGERPKGLSGGVPGPARRRVVCSGGDLPEPPEPGLLPNGTVTLLLSNNKITGLRNGSFLGLSLLEKLDLRNNIISTVQPGAFLGLGELKRLDLSNNRIGCLTSETFQGLPRLLRLNISGNIFSSLQPGVFDELPALKVVDLGTEFLTCDCHLRWLLPWAQNRSLQLSEHTLCAYPSALHAQALGSLQEAQLCCEGALELHTHHLIPSLRQVVFQGDRLPFQCSASYLGNDTRIRWYHNRAPVEGDEQAGILLAESLIHDCTFITSELTLSHIGVWASGEWECTVSMAQGNASKKVEIVVLETSASYCPAERVANNRGDFRWPRTLAGITAYQSCLQYPFTSVPLGGGAPGTRASRRCDRAGRWEPGDYSHCLYTNDITRVLYTFVLMPINASNALTLAHQLRVYTAEAASFSDMMDVVYVAQMIQKFLGYVDQIKELVEVMVDMASNLMLVDEHLLWLAQREDKACSRIVGALERIGGAALSPHAQHISVNARNVALEAYLIKPHSYVGLTCTAFQRREGGVPGTRPGSPGQNPPPEPEPPADQQLRFRCTTGRPNVSLSSFHIKNSVALASIQLPPSLFSSLPAALAPPVPPDCTLQLLVFRNGRLFHSHSNTSRPGAAGPGKRRGVATPVIFAGTSGCGVGNLTEPVAVSLRHWAEGAEPVAAWWSQEGPGEAGGWTSEGCQLRSSQPNVSALHCQHLGNVAVLMELSAFPREVGGAGAGLHPVVYPCTALLLLCLFATIITYILNHSSIRVSRKGWHMLLNLCFHIAMTSAVFAGGITLTNYQMVCQAVGITLHYSSLSTLLWMGVKARVLHKELTWRAPPPQEGDPALPTPSPMLRFYLIAGGIPLIICGITAAVNIHNYRDHSPYCWLVWRPSLGAFYIPVALILLITWIYFLCAGLRLRGPLAQNPKAGNSRASLEAGEELRGSTRLRGSGPLLSDSGSLLATGSARVGTPGPPEDGDSLYSPGVQLGALVTTHFLYLAMWACGALAVSQRWLPRVVCSCLYGVAASALGLFVFTHHCARRRDVRASWRACCPPASPAAPHAPPRALPAAAEDGSPVFGEGPPSLKSSPSGSSGHPLALGPCKLTNLQLAQSQVCEAGAAAGGEGEPEPAGTRGNLAHRHPNNVHHGRRAHKSRAKGHRAGEACGKNRLKALRGGAAGALELLSSESGSLHNSPTDSYLGSSRNSPGAGLQLEGEPMLTPSEGSDTSAAPLSEAGRAGQRRSASRDSLKGGGALEKESHRRSYPLNAASLNGAPKGGKYDDVTLMGAEVASGGCMKTGLWKSETTV

SEQ ID NO: 2 - protein, 971 aa, homo sapiens
MATVRASLRGALLLLLAVAGVAEVAGGLAPGSAGALCCNHSKDNQMCRDVCEQIFSSKSESRLKHLLQRAPDYCPETMVEIWNCMNSSLPGVFKKSDGWVGLGCCELAIALECRQACKQASSKNDISKVCRKEYENALFSCISRNEMGSVCCSYAGHHTNCREYCQAIFRTDSSPGPSQIKAVENYCASISPQLIHCVNNYTQSYPMRNPTDSLYCCDRAEDHACQNACKRILMSKKTEMEIVDGLIEGCKTQPLPQDPLWQCFLESSQSVHPGVTVHPPPSTGLDGAKLHCCSKANTSTCRELCTKLYSMSWGNTQSWQEFDRFCEYNPVEVSMLTCLADVREPCQLGCRNLTYCTNFNNRPTELFRSCNAQSDQGAMNDMKLWEKGSIKMPFINIPVLDIKKCQPEMWKAIACSLQIKPCHSKSRGSIICKSDCVEILKKCGDQNKFPEDHTAESICELLSPTDDLKNCIPLDTYLRPSTLGNIVEEVTHPCNPNPCPANELCEVNRKGCPSGDPCLPYFCVQGCKLGEASDFIVRQGTLIQVPSSAGEVGCYKICSCGQSGLLENCMEMHCIDLQKSCIVGGKRKSHGTSFSIDCNVCSCFAGNLVCSTRLCLSEHSSEDDRRTFTGLPCNCADQFVPVCGQNGRTYPSACIARCVGLQDHQFEFGSCMSKDPCNPNPCQKNQRCIPKPQVCLTTFDKFGCSQYECVPRQLACDQVQDPVCDTDHMEHNNLCTLYQRGKSLSYKGPCQPFCRATEPVCGHNGETYSSVCAAYSDRVAVDYYGDCQAVGVLSEHSSVAECASVKCPSLLAAGCKPIIPPGACCPLCAGMLRVLFDKEKLDTIAKVTNKKPITVLEILQKIRMHVSVPQCDVFGYFSIESEIVILIIPVDHYPKALQIEACNKEAEKIESLINSDSPTLASHVPLSALIISQVQVSSSVPSAGVRARPSCHSLLLPLSLGLALHLLWTYN

SEQ ID NO: 3 - protein, 1615 aa, homo sapiens
MEAAPPGPPWPLLLLLLLLLALCGCPAPAAASPLLLFANRRDVRLVDAGGVKLESTIVVSGLEDAAAVDFQFSKGAVYWTDVSEEAIKQTYLNQTGAAVQNVVISGLVSPDGLACDWVGKKLYWTDSETNRIEVANLNGTSRKVLFWQDLDQPRAIALDPAHGYMYWTDWGETPRIERAGMDGSTRKIIVDSDIYWPNGLTIDLEEQKLYWADAKLSFIHRANLDGSFRQKVVEGSLTHPFALTLSGDTLYWTDWQTRSIHACNKRTGGKRKEILSALYSPMDIQVLSQERQPFFHTRCEEDNGGCSHLCLLSPSEPFYTCACPTGVQLQDNGRTCKAGAEEVLLLARRTDLRRISLDTPDFTDIVLQVDDIRHAIAIDYDPLEGYVYWTDDEVRAIRRAYLDGSGAQTLVNTEINDPDGIAVDWVARNLYWTDTGTDRIEVTRLNGTSRKILVSEDLDEPRAIALHPVMGLMYWTDWGENPKIECANLDGQERRVLVNASLGWPNGLALDLQEGKLYWGDAKTDKIEVINVDGTKRRTLLEDKLPHIFGFTLLGDFIYWTDWQRRSIERVHKVKASRDVIIDQLPDLMGLKAVNVAKVVGTNPCADRNGGCSHLCFFTPHATRCGCPIGLELLSDMKTCIVPEAFLVFTSRAAIHRISLETNNNDVAIPLTGVKEASALDFDVSNNHIYWTDVSLKTISRAFMNGSSVEHVVEFGLDYPEGMAVDWMGKNLYWADTGTNRIEVARLDGQFRQVLVWRDLDNPRSLALDPTKGYIYWTEWGGKPRIVRAFMDGTNCMTLVDKVGRANDLTIDYADQRLYWTDLDTNMIESSNMLGQERVVIADDLPHPFGLTQYSDYIYWTDWNLHSIERADKTSGRNRTLIQGHLDFVMDILVFHSSRQDGLNDCMHNNGQCGQLCLAIPGGHRCGCASHYTLDPSSRNCSPPTTFLLFSQKSAISRMIPDDQHSPDLILPLHGLRNVKAIDYDPLDKFIYWVDGRQNIKRAKDDGTQPFVLTSLSQGQNPDRQPHDLSIDIYSRTLFWTCEATNTINVHRLSGEAMGVVLRGDRDKPRAIVVNAERGYLYFTNMQDRAAKIERAALDGTEREVLFTTGLIRPVALVVDNTLGKLFWVDADLKRIESCDLSGANRLTLEDANIVQPLGLTILGKHLYWIDRQQQMIERVEKTTGDKRTRIQGRVAHLTGIHAVEEVSLEEFSAHPCARDNGGCSHICIAKGDGTPRCSCPVHLVLLQNLLTCGEPPTCSPDQFACATGEIDCIPGAWRCDGFPECDDQSDEEGCPVCSAAQFPCARGQCVDLRLRCDGEADCQDRSDEADCDAICLPNQFRCASGQCVLIKQQCDSFPDCIDGSDELMCEITKPPSDDSPAHSSAIGPVIGIILSLFVMGGVYFVCQRVVCQRYAGANGPFPHEYVSGTPHVPLNFIAPGGSQHGPFTGIACGKSMMSSVSLMGGRGGVPLYDRNHVTGASSSSSSSTKATLYPPILNPPPSPATDPSLYNMDMFYSSNIPATARPYRPYIIRGMAPPTTPCSTDVCDSDYSASRWKASKYYLDLNSDSDPYPPPPTPHSQYLSAEDSCPPSPATERSYFHLFPPPPSPCTDSS

SEQ ID NO: 4 - protein, 1613 aa, homo sapiens
MGAVLRSLLACSFCVLLRAAPLLLYANRRDLRLVDATNGKENATIVVGGLEDAAAVDFVFSHGLIYWSDVSEEAIKRTEFNKTESVQNVVVSGLLSPDGLACDWLGEKLYWTDSETNRIEVSNLDGSLRKVLFWQELDQPRAIALDPSSGFMYWTDWGEVPKIERAGMDGSSRFIIINSEIYWPNGLTLDYEEQKLYWADAKLNFIHKSNLDGTNRQAVVKGSLPHPFALTLFEDILYWTDWSTHSILACNKYTGEGLREIHSDIFSPMDIHAFSQQRQPNATNPCGIDNGGCSHLCLMSPVKPFYQCACPTGVKLLENGKTCKDGATELLLLARRTDLRRISLDTPDFTDIVLQLEDIRHAIAIDYDPVEGYIYWTDDEVRAIRRSFIDGSGSQFVVTAQIAHPDGIAVDWVARNLYWTDTGTDRIEVTRLNGTMRKILISEDLEEPRAIVLDPMVGYMYWTDWGEIPKIERAALDGSDRVVLVNTSLGWPNGLALDYDEGKIYWGDAKTDKIEVMNTDGTGRRVLVEDKIPHIFGFTLLGDYVYWTDWQRRSIERVHKRSAEREVIIDQLPDLMGLKATNVHRVIGSNPCAEENGGCSHLCLYRPQGLRCACPIGFELISDMKTCIVPEAFLLFSRRADIRRISLETNNNNVAIPLTGVKEASALDFDVTDNRIYWTDISLKTISRAFMNGSALEHVVEFGLDYPEGMAVDWLGKNLYWADTGTNRIEVSKLDGQHRQVLVWKDLDSPRALALDPAEGFMYWTEWGGKPKIDRAAMDGSERTTLVPNVGRANGLTIDYAKRRLYWTDLDTNLIESSNMLGLNREVIADDLPHPFGLTQYQDYIYWTDWSRRSIERANKTSGQNRTIIQGHLDYVMDILVFHSSRQSGWNECASSNGHCSHLCLAVPVGGFVCGCPAHYSLNADNRTCSAPTTFLLFSQKSAINRMVIDEQQSPDIILPIHSLRNVRAIDYDPLDKQLYWIDSRQNMIRKAQEDGSQGFTVVVSSVPSQNLEIQPYDLSIDIYSRYIYWTCEATNVINVTRLDGRSVGVVLKGEQDRPRAVVVNPEKGYMYFTNLQERSPKIERAALDGTEREVLFFSGLSKPIALALDSRLGKLFWADSDLRRIESSDLSGANRIVLEDSNILQPVGLTVFENWLYWIDKQQQMIEKIDMTGREGRTKVQARIAQLSDIHAVKELNLQEYRQHPCAQDNGGCSHICLVKGDGTTRCSCPMHLVLLQDELSCGEPPTCSPQQFTCFTGEIDCIPVAWRCDGFTECEDHSDELNCPVCSESQFQCASGQCIDGALRCNGDANCQDKSDEKNCEVLCLIDQFRCANGQCIGKHKKCDHNVDCSDKSDELDCYPTEEPAPQATNTVGSVIGVIVTIFVSGTVYFICQRMLCPRMKGDGETMTNDYVVHGPASVPLGYVPHPSSLSGSLPGMSRGKSMISSLSIMGGSSGPPYDRAHVTGASSSSSSSTKGTYFPAILNPPPSPATERSHYTMEFGYSSNSPSTHRSYSYRPYSYRHFAPPTTPCSTDVCDSDYAPSRRMTSVATAKGYTSDLNYDSEPVPPPPTPRSQYLSAEENYESCPPSPYTERSYSHHLYPPPPSPCTDSS

SEQ ID NO: 5 - protein, 48 aa, homo sapiens
CCDRAEDHACQNACKRILMSKKTEMEIVDGLIEGCKTQPLPQDPLWQC

SEQ ID NO: 6 - protein, 47 aa, homo sapiens
CCSKANTSTCRELCTKLYSMSWGNTQSWQEFDRFCEYNPVEVSMLTC

SEQ ID NO: 7 - protein, 6 aa, artificial sequence
  fragment of Frizzled receptor
  SITE (3)..(5): any amino acid
KTXXXW

SEQ ID NO: 8 - protein, 4 aa, artificial sequence
  LRP repeat domain
YWTD

SEQ ID NO: 9 - protein, 4 aa, artificial sequence
  LRP motif
  SITE (3)..(3): any amino acid
NPXY

SEQ ID NO: 10 - protein, 5 aa, artificial sequence
  LRP motif
PPPSP

SEQ ID NO: 11 - protein, 16 aa, artificial sequence
  Frizzled-binding domain
  SITE (1)..(1): any amino acid
  SITE (3)..(6): any amino acid
  SITE (9)..(15): any amino acid
XKXXXXSGXXXXXXXW

SEQ ID NO: 12 - protein, 16 aa, homo sapiens
CKCHGVSGSCTTKTCW

SEQ ID NO: 13 - protein, 5 aa, artificial sequence
  Frizzled-binding domain
  SITE (2)..(2): any amino acid
  SITE (4)..(4): any amino acid
WXCXV

SEQ ID NO: 14 - protein, 89 aa, homo sapiens
MYHTKGQEGSVCLRSSDCASGLCCARHFWSKICKPVLKEGQVCTKHRRKGSHGLEIFQRCYCGEGLSCRIQKDHHQASNSSRLHTCQRH

SEQ ID NO: 15 - protein, 349 aa, homo sapiens
MNRKARRCLGHLFLSLGMVYLRIGGFSSVVALGASIICNKIPGLAPRQRAICQSRPDAIIVIGEGSQMGLDECQFQFRNGRWNCSALGERTVFGKELKVGSREAAFTYAIIAAGVAHAITAACTQGNLSDCGCDKEKQGQYHRDEGWKWGGCSADIRYGIGFAKVFVDAREIKQNARTLMNLHNNEAGRKILEENMKLECKCHGVSGSCTTKTCWTTLPQFRELGYVLKDKYNEAVHVEPVRASRNKRPTFLKIKKPLSYRKPMDTDLVYIEKSPNYCEEDPVTGSVGTQGRACNKTAPQASGCDLMCCGRGYNTHQYARVWQCNCKFHWCCYVKCNTCSERTEMYTCK

SEQ ID NO: 16 - protein, 349 aa, homo sapiens
MHRNFRKWIFYVFLCFGVLYVKLGALSSVVALGANIICNKIPGLAPRQRAICQSRPDAIIVIGEGAQMGINECQYQFRFGRWNCSALGEKTVFGQELRVGSREAAFTYAITAAGVAHAVTAACSQGNLSNCGCDREKQGYYNQAEGWKWGGCSADVRYGIDFSRRFVDAREIKKNARRLMNLHNNEAGRKVLEDRMQLECKCHGVSGSCTTKTCWTTLPKFREVGHLLKEKYNAAVQVEVVRASRLRQPTFLRIKQLRSYQKPMETDLVYIEKSPNYCEEDAATGSVGTQGRLCNRTSPGADGCDTMCCGRGYNTHQYTKVWQCNCKFHWCCFVKCNTCSERTEVFTCK

SEQ ID NO: 17 - protein, 42 aa, homo sapiens
HVEPVRASRNKRPTFLKIKKPLSYRKPMDTDLVYIEKSPNYC

SEQ ID NO: 18 - protein, 29 aa, homo sapiens
VEPVRASRNKRPTFLKIKKPLSYRKPMDT

SEQ ID NO: 19 - protein, 29 aa, homo sapiens
VEVVRASRLRQPTFLRIKQLRSYQKPMET

SEQ ID NO: 20 - protein, 29 aa, artificial sequence
  RECK-binding domain
  SITE (1)..(3): any amino acid
  SITE (5)..(5): any amino acid
  SITE (7)..(7): any amino acid
  SITE (9)..(13): any amino acid
  SITE (16)..(16): any amino acid
  SITE (18)..(22): any amino acid
  SITE (24)..(24): any amino acid
  SITE (26)..(29): any amino acid
XXXVXAXRXXXXXFLXIXXXXXYXKXXXX

SEQ ID NO: 21 - protein, 22 aa, artificial sequence
  RECK-binding domain
  SITE (2)..(2): any amino acid
  SITE (4)..(4): any amino acid
  SITE (6)..(10): any amino acid
  SITE (13)..(13): any amino acid
  SITE (15)..(19): any amino acid
  SITE (21)..(21): any amino acid
VXAXRXXXXXFLXIXXXXXYXK

SEQ ID NO: 22 - protein, 29 aa, artificial sequence
  RECK-binding domain
  SITE (1)..(3): any amino acid
  SITE (5)..(5): any amino acid
  SITE (7)..(7): any amino acid
  SITE (9)..(13): any amino acid
  SITE (16)..(24): any amino acid
  SITE (26)..(29): any amino acid
XXXVXAXRXXXXXFLXXXXXXXXXKXXXX

SEQ ID NO: 23 - protein, 22 aa, artificial sequence
  RECK-binding domain
  SITE (2)..(2): any amino acid
  SITE (4)..(4): any amino acid
  SITE (6)..(10): any amino acid
  SITE (13)..(21): any amino acid
VXAXRXXXXXFLXXXXXXXXXK

SEQ ID NO: 24 - protein, 247 aa, artificial sequence
  N-terminal domain (NTD) of human Wnt7a polypeptide
LGASIICNKIPGLAPRQRAICQSRPDAIIVIGEGSQMGLDECQFQFRNGRWNCSALGERTVFGKELKVGSREAAFTYAIIAAGVAHAITAACTQGNLSDCGCDKEKQGQYHRDEGWKWGGCSADIRYGIGFAKVFVDAREIKQNARTLMNLHNNEAGRKILEENMKLECKCHGVSGSCTTKTCWTTLPQFRELGYVLKDKYNEAVHVEPVRASRNKRPTFLKIKKPLSYRKPMDTDLVYIEKSPNYC

SEQ ID NO: 25 - protein, 247 aa, artificial sequence
  N-terminal domain (NTD) of human Wnt7b polypeptide
LGANIICNKIPGLAPRQRAICQSRPDAIIVIGEGAQMGINECQYQFRFGRWNCSALGEKTVFGQELRVGSREAAFTYAITAAGVAHAVTAACSQGNLSNCGCDREKQGYYNQAEGWKWGGCSADVRYGIDFSRRFVDAREIKKNARRLMNLHNNEAGRKVLEDRMQLECKCHGVSGSCTTKTCWTTLPKFREVGHLLKEKYNAAVQVEVVRASRLRQPTFLRIKQLRSYQKPMETDLVYIEKSPNYC

SEQ ID NO: 26 - protein, 31 aa, artificial sequence
  signal peptide human Wnt7a polypeptide
MNRKARRCLGHLFLSLGMVYLRIGGFSSVVA

SEQ ID NO: 27 - protein, 31 aa, artificial sequence
  signal peptide human Wnt7b polypeptide
MHRNFRKWIFYVFLCFGVLYVKLGALSSVVA

SEQ ID NO: 28 - protein, 247 aa, artificial sequence
  human N-terminal domain (NTD) Wnt7a variant K159A
LGASIICNKIPGLAPRQRAICQSRPDAIIVIGEGSQMGLDECQFQFRNGRWNCSALGERTVFGKELKVGSREAAFTYAIIAAGVAHAITAACTQGNLSDCGCDKEKQGQYHRDEGWKWGGCSADIRYGIGFAKVFVDAREIKQNARTLMNLHNNEAGRAILEENMKLECKCHGVSGSCTTKTCWTTLPQFRELGYVLKDKYNEAVHVEPVRASRNKRPTFLKIKKPLSYRKPMDTDLVYIEKSPNYC

SEQ ID NO: 29 - protein, 247 aa, artificial sequence
  human N-terminal domain (NTD) Wnt7a variant A27R
LGASIICNKIPGLAPRQRAICQSRPDRIIVIGEGSQMGLDECQFQFRNGRWNCSALGERTVFGKELKVGSREAAFTYAIIAAGVAHAITAACTQGNLSDCGCDKEKQGQYHRDEGWKWGGCSADIRYGIGFAKVFVDAREIKQNARTLMNLHNNEAGRKILEENMKLECKCHGVSGSCTTKTCWTTLPQFRELGYVLKDKYNEAVHVEPVRASRNKRPTFLKIKKPLSYRKPMDTDLVYIEKSPNYC

SEQ ID NO: 30 - protein, 247 aa, artificial sequence
  human N-terminal domain (NTD) Wnt7a variant E33A
LGASIICNKIPGLAPRQRAICQSRPDAIIVIGAGSQMGLDECQFQFRNGRWNCSALGERTVFGKELKVGSREAAFTYAIIAAGVAHAITAACTQGNLSDCGCDKEKQGQYHRDEGWKWGGCSADIRYGIGFAKVFVDAREIKQNARTLMNLHNNEAGRKILEENMKLECKCHGVSGSCTTKTCWTTLPQFRELGYVLKDKYNEAVHVEPVRASRNKRPTFLKIKKPLSYRKPMDTDLVYIEKSPNYC

SEQ ID NO: 31 - protein, 247 aa, artificial sequence
  human N-terminal domain (NTD)  Wnt7a variant E41A
LGASIICNKIPGLAPRQRAICQSRPDAIIVIGEGSQMGLDACQFQFRNGRWNCSALGERTVFGKELKVGSREAAFTYAIIAAGVAHAITAACTQGNLSDCGCDKEKQGQYHRDEGWKWGGCSADIRYGIGFAKVFVDAREIKQNARTLMNLHNNEAGRKILEENMKLECKCHGVSGSCTTKTCWTTLPQFRELGYVLKDKYNEAVHVEPVRASRNKRPTFLKIKKPLSYRKPMDTDLVYIEKSPNYC

SEQ ID NO: 32 - protein, 247 aa, artificial sequence
  human N-terminal domain (NTD)  Wnt7a variant F44A
LGASIICNKIPGLAPRQRAICQSRPDAIIVIGEGSQMGLDECQAQFRNGRWNCSALGERTVFGKELKVGSREAAFTYAIIAAGVAHAITAACTQGNLSDCGCDKEKQGQYHRDEGWKWGGCSADIRYGIGFAKVFVDAREIKQNARTLMNLHNNEAGRKILEENMKLECKCHGVSGSCTTKTCWTTLPQFRELGYVLKDKYNEAVHVEPVRASRNKRPTFLKIKKPLSYRKPMDTDLVYIEKSPNYC

SEQ ID NO: 33 - protein, 247 aa, artificial sequence
  human N-terminal domain (NTD)  Wnt7a variant N52Q
LGASIICNKIPGLAPRQRAICQSRPDAIIVIGEGSQMGLDECQFQFRNGRWQCSALGERTVFGKELKVGSREAAFTYAIIAAGVAHAITAACTQGNLSDCGCDKEKQGQYHRDEGWKWGGCSADIRYGIGFAKVFVDAREIKQNARTLMNLHNNEAGRKILEENMKLECKCHGVSGSCTTKTCWTTLPQFRELGYVLKDKYNEAVHVEPVRASRNKRPTFLKIKKPLSYRKPMDTDLVYIEKSPNYC

SEQ ID NO: 34 - protein, 247 aa, artificial sequence
  human N-terminal domain (NTD)  Wnt7a variant I129A
LGASIICNKIPGLAPRQRAICQSRPDAIIVIGEGSQMGLDECQFQFRNGRWNCSALGERTVFGKELKVGSREAAFTYAIIAAGVAHAITAACTQGNLSDCGCDKEKQGQYHRDEGWKWGGCSADIRYGAGFAKVFVDAREIKQNARTLMNLHNNEAGRKILEENMKLECKCHGVSGSCTTKTCWTTLPQFRELGYVLKDKYNEAVHVEPVRASRNKRPTFLKIKKPLSYRKPMDTDLVYIEKSPNYC

SEQ ID NO: 35 - protein, 247 aa, artificial sequence
  human N-terminal domain (NTD)  Wnt7a variant F131A
LGASIICNKIPGLAPRQRAICQSRPDAIIVIGEGSQMGLDECQFQFRNGRWNCSALGERTVFGKELKVGSREAAFTYAIIAAGVAHAITAACTQGNLSDCGCDKEKQGQYHRDEGWKWGGCSADIRYGIGAAKVFVDAREIKQNARTLMNLHNNEAGRKILEENMKLECKCHGVSGSCTTKTCWTTLPQFRELGYVLKDKYNEAVHVEPVRASRNKRPTFLKIKKPLSYRKPMDTDLVYIEKSPNYC

SEQ ID NO: 36 - protein, 247 aa, artificial sequence
  human N-terminal domain (NTD) Wnt7a variant K133A
LGASIICNKIPGLAPRQRAICQSRPDAIIVIGEGSQMGLDECQFQFRNGRWNCSALGERTVFGKELKVGSREAAFTYAIIAAGVAHAITAACTQGNLSDCGCDKEKQGQYHRDEGWKWGGCSADIRYGIGFAAVFVDAREIKQNARTLMNLHNNEAGRKILEENMKLECKCHGVSGSCTTKTCWTTLPQFRELGYVLKDKYNEAVHVEPVRASRNKRPTFLKIKKPLSYRKPMDTDLVYIEKSPNYC

SEQ ID NO: 37 - protein, 247 aa, artificial sequence
  human N-terminal domain (NTD) Wnt7a variant I141A
LGASIICNKIPGLAPRQRAICQSRPDAIIVIGEGSQMGLDECQFQFRNGRWNCSALGERTVFGKELKVGSREAAFTYAIIAAGVAHAITAACTQGNLSDCGCDKEKQGQYHRDEGWKWGGCSADIRYGIGFAKVFVDAREAKQNARTLMNLHNNEAGRKILEENMKLECKCHGVSGSCTTKTCWTTLPQFRELGYVLKDKYNEAVHVEPVRASRNKRPTFLKIKKPLSYRKPMDTDLVYIEKSPNYC

SEQ ID NO: 38 - protein, 247 aa, artificial sequence
  human N-terminal domain (NTD) Wnt7a variant R158A
LGASIICNKIPGLAPRQRAICQSRPDAIIVIGEGSQMGLDECQFQFRNGRWNCSALGERTVFGKELKVGSREAAFTYAIIAAGVAHAITAACTQGNLSDCGCDKEKQGQYHRDEGWKWGGCSADIRYGIGFAKVFVDAREIKQNARTLMNLHNNEAGAKILEENMKLECKCHGVSGSCTTKTCWTTLPQFRELGYVLKDKYNEAVHVEPVRASRNKRPTFLKIKKPLSYRKPMDTDLVYIEKSPNYC

SEQ ID NO: 39 - protein, 247 aa, artificial sequence
  human N-terminal domain (NTD) Wnt7a variant K181A
LGASIICNKIPGLAPRQRAICQSRPDAIIVIGEGSQMGLDECQFQFRNGRWNCSALGERTVFGKELKVGSREAAFTYAIIAAGVAHAITAACTQGNLSDCGCDKEKQGQYHRDEGWKWGGCSADIRYGIGFAKVFVDAREIKQNARTLMNLHNNEAGRKILEENMKLECKCHGVSGSCTTATCWTTLPQFRELGYVLKDKYNEAVHVEPVRASRNKRPTFLKIKKPLSYRKPMDTDLVYIEKSPNYC

SEQ ID NO: 40 - protein, 247 aa, artificial sequence
  human N-terminal domain (NTD) Wnt7a variant R191A
LGASIICNKIPGLAPRQRAICQSRPDAIIVIGEGSQMGLDECQFQFRNGRWNCSALGERTVFGKELKVGSREAAFTYAIIAAGVAHAITAACTQGNLSDCGCDKEKQGQYHRDEGWKWGGCSADIRYGIGFAKVFVDAREIKQNARTLMNLHNNEAGRKILEENMKLECKCHGVSGSCTTKTCWTTLPQFAELGYVLKDKYNEAVHVEPVRASRNKRPTFLKIKKPLSYRKPMDTDLVYIEKSPNYC

SEQ ID NO: 41 - protein, 247 aa, artificial sequence
  human N-terminal domain (NTD) Wnt7a variant K198A
LGASIICNKIPGLAPRQRAICQSRPDAIIVIGEGSQMGLDECQFQFRNGRWNCSALGERTVFGKELKVGSREAAFTYAIIAAGVAHAITAACTQGNLSDCGCDKEKQGQYHRDEGWKWGGCSADIRYGIGFAKVFVDAREIKQNARTLMNLHNNEAGRKILEENMKLECKCHGVSGSCTTKTCWTTLPQFRELGYVLADKYNEAVHVEPVRASRNKRPTFLKIKKPLSYRKPMDTDLVYIEKSPNYC

SEQ ID NO: 42 - protein, 247 aa, artificial sequence
  human N-terminal domain (NTD) Wnt7a variant V205A
LGASIICNKIPGLAPRQRAICQSRPDAIIVIGEGSQMGLDECQFQFRNGRWNCSALGERTVFGKELKVGSREAAFTYAIIAAGVAHAITAACTQGNLSDCGCDKEKQGQYHRDEGWKWGGCSADIRYGIGFAKVFVDAREIKQNARTLMNLHNNEAGRKILEENMKLECKCHGVSGSCTTKTCWTTLPQFRELGYVLKDKYNEAAHVEPVRASRNKRPTFLKIKKPLSYRKPMDTDLVYIEKSPNYC

SEQ ID NO: 43 - protein, 247 aa, artificial sequence
  human N-terminal domain (NTD) Wnt7a variant E208A
LGASIICNKIPGLAPRQRAICQSRPDAIIVIGEGSQMGLDECQFQFRNGRWNCSALGERTVFGKELKVGSREAAFTYAIIAAGVAHAITAACTQGNLSDCGCDKEKQGQYHRDEGWKWGGCSADIRYGIGFAKVFVDAREIKQNARTLMNLHNNEAGRKILEENMKLECKCHGVSGSCTTKTCWTTLPQFRELGYVLKDKYNEAVHVAPVRASRNKRPTFLKIKKPLSYRKPMDTDLVYIEKSPNYC

SEQ ID NO: 44 - protein, 247 aa, artificial sequence
  human N-terminal domain (NTD) Wnt7a variant K216A
LGASIICNKIPGLAPRQRAICQSRPDAIIVIGEGSQMGLDECQFQFRNGRWNCSALGERTVFGKELKVGSREAAFTYAIIAAGVAHAITAACTQGNLSDCGCDKEKQGQYHRDEGWKWGGCSADIRYGIGFAKVFVDAREIKQNARTLMNLHNNEAGRKILEENMKLECKCHGVSGSCTTKTCWTTLPQFRELGYVLKDKYNEAVHVEPVRASRNARPTFLKIKKPLSYRKPMDTDLVYIEKSPNYC

SEQ ID NO: 45 - protein, 247 aa, artificial sequence
  human N-terminal domain (NTD) Wnt7a variant K222A
LGASIICNKIPGLAPRQRAICQSRPDAIIVIGEGSQMGLDECQFQFRNGRWNCSALGERTVFGKELKVGSREAAFTYAIIAAGVAHAITAACTQGNLSDCGCDKEKQGQYHRDEGWKWGGCSADIRYGIGFAKVFVDAREIKQNARTLMNLHNNEAGRKILEENMKLECKCHGVSGSCTTKTCWTTLPQFRELGYVLKDKYNEAVHVEPVRASRNKRPTFLAIKKPLSYRKPMDTDLVYIEKSPNYC

SEQ ID NO: 46 - protein, 247 aa, artificial sequence
  human N-terminal domain (NTD) Wnt7a variant I223A
LGASIICNKIPGLAPRQRAICQSRPDAIIVIGEGSQMGLDECQFQFRNGRWNCSALGERTVFGKELKVGSREAAFTYAIIAAGVAHAITAACTQGNLSDCGCDKEKQGQYHRDEGWKWGGCSADIRYGIGFAKVFVDAREIKQNARTLMNLHNNEAGRKILEENMKLECKCHGVSGSCTTKTCWTTLPQFRELGYVLKDKYNEAVHVEPVRASRNKRPTFLKAKKPLSYRKPMDTDLVYIEKSPNYC

SEQ ID NO: 47 - protein, 247 aa, artificial sequence
  human N-terminal domain (NTD) Wnt7a variant Y229A
LGASIICNKIPGLAPRQRAICQSRPDAIIVIGEGSQMGLDECQFQFRNGRWNCSALGERTVFGKELKVGSREAAFTYAIIAAGVAHAITAACTQGNLSDCGCDKEKQGQYHRDEGWKWGGCSADIRYGIGFAKVFVDAREIKQNARTLMNLHNNEAGRKILEENMKLECKCHGVSGSCTTKTCWTTLPQFRELGYVLKDKYNEAVHVEPVRASRNKRPTFLKIKKPLSARKPMDTDLVYIEKSPNYC

SEQ ID NO: 48 - protein, 247 aa, artificial sequence
  human N-terminal domain (NTD) Wnt7a variant P232A
LGASIICNKIPGLAPRQRAICQSRPDAIIVIGEGSQMGLDECQFQFRNGRWNCSALGERTVFGKELKVGSREAAFTYAIIAAGVAHAITAACTQGNLSDCGCDKEKQGQYHRDEGWKWGGCSADIRYGIGFAKVFVDAREIKQNARTLMNLHNNEAGRKILEENMKLECKCHGVSGSCTTKTCWTTLPQFRELGYVLKDKYNEAVHVEPVRASRNKRPTFLKIKKPLSYRKAMDTDLVYIEKSPNYC

SEQ ID NO: 49 - protein, 247 aa, artificial sequence
  human N-terminal domain (NTD) Wnt7a variant T235A
LGASIICNKIPGLAPRQRAICQSRPDAIIVIGEGSQMGLDECQFQFRNGRWNCSALGERTVFGKELKVGSREAAFTYAIIAAGVAHAITAACTQGNLSDCGCDKEKQGQYHRDEGWKWGGCSADIRYGIGFAKVFVDAREIKQNARTLMNLHNNEAGRKILEENMKLECKCHGVSGSCTTKTCWTTLPQFRELGYVLKDKYNEAVHVEPVRASRNKRPTFLKIKKPLSYRKPMDADLVYIEKSPNYC

SEQ ID NO: 50 - protein, 318 aa, artificial sequence
  human full Wnt7a variant E248A
LGASIICNKIPGLAPRQRAICQSRPDAIIVIGEGSQMGLDECQFQFRNGRWNCSALGERTVFGKELKVGSREAAFTYAIIAAGVAHAITAACTQGNLSDCGCDKEKQGQYHRDEGWKWGGCSADIRYGIGFAKVFVDAREIKQNARTLMNLHNNEAGRKILEENMKLECKCHGVSGSCTTKTCWTTLPQFRELGYVLKDKYNEAVHVEPVRASRNKRPTFLKIKKPLSYRKPMDTDLVYIEKSPNYCAEDPVTGSVGTQGRACNKTAPQASGCDLMCCGRGYNTHQYARVWQCNCKFHWCCYVKCNTCSERTEMYTCK

SEQ ID NO: 51 - protein, 318 aa, homo sapiens
LGASIICNKIPGLAPRQRAICQSRPDAIIVIGEGSQMGLDECQFQFRNGRWNCSALGERTVFGKELKVGSREAAFTYAIIAAGVAHAITAACTQGNLSDCGCDKEKQGQYHRDEGWKWGGCSADIRYGIGFAKVFVDAREIKQNARTLMNLHNNEAGRKILEENMKLECKCHGVSGSCTTKTCWTTLPQFRELGYVLKDKYNEAVHVEPVRASRNKRPTFLKIKKPLSYRKPMDTDLVYIEKSPNYCEEDPVTGSVGTQGRACNKTAPQASGCDLMCCGRGYNTHQYARVWQCNCKFHWCCYVKCNTCSERTEMYTCK

SEQ ID NO: 52 - protein, 318 aa, artificial sequence
  human full Wnt7a variant R289A
LGASIICNKIPGLAPRQRAICQSRPDAIIVIGEGSQMGLDECQFQFRNGRWNCSALGERTVFGKELKVGSREAAFTYAIIAAGVAHAITAACTQGNLSDCGCDKEKQGQYHRDEGWKWGGCSADIRYGIGFAKVFVDAREIKQNARTLMNLHNNEAGRKILEENMKLECKCHGVSGSCTTKTCWTTLPQFRELGYVLKDKYNEAVHVEPVRASRNKRPTFLKIKKPLSYRKPMDTDLVYIEKSPNYCEEDPVTGSVGTQGRACNKTAPQASGCDLMCCGRGYNTHQYAAVWQCNCKFHWCCYVKCNTCSERTEMYTCK

SEQ ID NO: 53 - protein, 318 aa, artificial sequence
  human full Wnt7a variant W291A
LGASIICNKIPGLAPRQRAICQSRPDAIIVIGEGSQMGLDECQFQFRNGRWNCSALGERTVFGKELKVGSREAAFTYAIIAAGVAHAITAACTQGNLSDCGCDKEKQGQYHRDEGWKWGGCSADIRYGIGFAKVFVDAREIKQNARTLMNLHNNEAGRKILEENMKLECKCHGVSGSCTTKTCWTTLPQFRELGYVLKDKYNEAVHVEPVRASRNKRPTFLKIKKPLSYRKPMDTDLVYIEKSPNYCEEDPVTGSVGTQGRACNKTAPQASGCDLMCCGRGYNTHQYARVAQCNCKFHWCCYVKCNTCSERTEMYTCK

SEQ ID NO: 54 - protein, 318 aa, artificial sequence
  human full Wnt7a variant T307A
LGASIICNKIPGLAPRQRAICQSRPDAIIVIGEGSQMGLDECQFQFRNGRWNCSALGERTVFGKELKVGSREAAFTYAIIAAGVAHAITAACTQGNLSDCGCDKEKQGQYHRDEGWKWGGCSADIRYGIGFAKVFVDAREIKQNARTLMNLHNNEAGRKILEENMKLECKCHGVSGSCTTKTCWTTLPQFRELGYVLKDKYNEAVHVEPVRASRNKRPTFLKIKKPLSYRKPMDTDLVYIEKSPNYCEEDPVTGSVGTQGRACNKTAPQASGCDLMCCGRGYNTHQYARVWQCNCKFHWCCYVKCNACSERTEMYTCK

SEQ ID NO: 55 - protein, 11 aa, artificial sequence
  peptide displayed on AAV-PHP.B
SAQTLAVPFKA

SEQ ID NO: 56 - protein, 11 aa, artificial sequence
  peptide displayed on AAV-PHP.eB
SDGTLAVPFKA

SEQ ID NO: 57 - protein, 7 aa, artificial sequence
  peptide displayed on AAV-BR1
NRGTEWD

SEQ ID NO: 58 - protein, 27 aa, artificial sequence
  xenopus Levis
VEPVRASRNKRPTFLKIKNSYRKPMDT

SEQ ID NO: 59 - protein, 29 aa, artificial sequence
  danio rerio
VEPVRASRNKRPAFLKVKKPYSYRKPMDT

SEQ ID NO: 60 - protein, 29 aa, artificial sequence
  danio rerio
VEPVKATRHKRPTFLKIKKPYSYRKPMDT

SEQ ID NO: 61 - protein, 29 aa, artificial sequence
  mus musculus
VEVVRASRLRQPTFLRIKQLRSYQKPMET

SEQ ID NO: 62 - protein, 29 aa, artificial sequence
  gallus gallus
VEVVRASRLRQPTFLKIKQIKSYQKPMET

SEQ ID NO: 63 - protein, 29 aa, artificial sequence
  xenopus Levis
VEVVRANRLRQPTFLKIKKVRSYQKPMET

SEQ ID NO: 64 - protein, 28 aa, artificial sequence
  Danio rerio
VEVVRASRLRQPTFLKVKRTRHQKPLET

SEQ ID NO: 65 - protein, 29 aa, artificial sequence
  Danio rerio
VEAVRATRFRQPSFLRLKQSRGYIKPTDT

SEQ ID NO: 66 - protein, 29 aa, artificial sequence
  mus musculus
MVVEKHRESRGWVETLRPRYTYFKVPTER

SEQ ID NO: 67 - protein, 29 aa, artificial sequence
  quadruple pWnt7a4A variant
VEPARASRNKRPTAAKIKKPLSYRAPMDT

SEQ ID NO: 68 - protein, 247 aa, artificial sequence
  human N-terminal domain (NTD) Wnt7a variant Q17A
LGASIICNKIPGLAPRARAICQSRPDAIIVIGEGSQMGLDECQFQFRNGRWNCSALGERTVFGKELKVGSREAAFTYAIIAAGVAHAITAACTQGNLSDCGCDKEKQGQYHRDEGWKWGGCSADIRYGIGFAKVFVDAREIKQNARTLMNLHNNEAGRKILEENMKLECKCHGVSGSCTTKTCWTTLPQFRELGYVLKDKYNEAVHVEPVRASRNKRPTFLKIKKPLSYRKPMDTDLVYIEKSPNYC

SEQ ID NO: 69 - protein, 247 aa, artificial sequence
  human N-terminal domain (NTD) Wnt7a variant I20A
LGASIICNKIPGLAPRQRAACQSRPDAIIVIGEGSQMGLDECQFQFRNGRWNCSALGERTVFGKELKVGSREAAFTYAIIAAGVAHAITAACTQGNLSDCGCDKEKQGQYHRDEGWKWGGCSADIRYGIGFAKVFVDAREIKQNARTLMNLHNNEAGRKILEENMKLECKCHGVSGSCTTKTCWTTLPQFRELGYVLKDKYNEAVHVEPVRASRNKRPTFLKIKKPLSYRKPMDTDLVYIEKSPNYC

SEQ ID NO: 70 - protein, 247 aa, artificial sequence
  human N-terminal domain (NTD) Wnt7a variant P25A
LGASIICNKIPGLAPRQRAICQSRADAIIVIGEGSQMGLDECQFQFRNGRWNCSALGERTVFGKELKVGSREAAFTYAIIAAGVAHAITAACTQGNLSDCGCDKEKQGQYHRDEGWKWGGCSADIRYGIGFAKVFVDAREIKQNARTLMNLHNNEAGRKILEENMKLECKCHGVSGSCTTKTCWTTLPQFRELGYVLKDKYNEAVHVEPVRASRNKRPTFLKIKKPLSYRKPMDTDLVYIEKSPNYC

SEQ ID NO: 71 - protein, 247 aa, artificial sequence
  human N-terminal domain (NTD) Wnt7a variant M37A
LGASIICNKIPGLAPRQRAICQSRPDAIIVIGEGSQAGLDECQFQFRNGRWNCSALGERTVFGKELKVGSREAAFTYAIIAAGVAHAITAACTQGNLSDCGCDKEKQGQYHRDEGWKWGGCSADIRYGIGFAKVFVDAREIKQNARTLMNLHNNEAGRKILEENMKLECKCHGVSGSCTTKTCWTTLPQFRELGYVLKDKYNEAVHVEPVRASRNKRPTFLKIKKPLSYRKPMDTDLVYIEKSPNYC

SEQ ID NO: 72 - protein, 247 aa, artificial sequence
  human N-terminal domain (NTD) Wnt7a variant L39A
LGASIICNKIPGLAPRQRAICQSRPDAIIVIGEGSQMGADECQFQFRNGRWNCSALGERTVFGKELKVGSREAAFTYAIIAAGVAHAITAACTQGNLSDCGCDKEKQGQYHRDEGWKWGGCSADIRYGIGFAKVFVDAREIKQNARTLMNLHNNEAGRKILEENMKLECKCHGVSGSCTTKTCWTTLPQFRELGYVLKDKYNEAVHVEPVRASRNKRPTFLKIKKPLSYRKPMDTDLVYIEKSPNYC

SEQ ID NO: 73 - DNA, 25 bp, artificial sequence
  wnt7aa Morpholino
ttccatttgaccctacttacccaat

SEQ ID NO: 74 - protein, 247 aa, artificial sequence
  human N-terminal domain (NTD) Wnt7a variant I28A
LGASIICNKIPGLAPRQRAICQSRPDAAIVIGEGSQMGLDECQFQFRNGRWNCSALGERTVFGKELKVGSREAAFTYAIIAAGVAHAITAACTQGNLSDCGCDKEKQGQYHRDEGWKWGGCSADIRYGIGFAKVFVDAREIKQNARTLMNLHNNEAGRKILEENMKLECKCHGVSGSCTTKTCWTTLPQFRELGYVLKDKYNEAVHVEPVRASRNKRPTFLKIKKPLSYRKPMDTDLVYIEKSPNYC

SEQ ID NO: 75 - protein, 247 aa, artificial sequence
  human N-terminal domain (NTD) Wnt7a variant R50A
LGASIICNKIPGLAPRQRAICQSRPDAIIVIGEGSQMGLDECQFQFRNGAWNCSALGERTVFGKELKVGSREAAFTYAIIAAGVAHAITAACTQGNLSDCGCDKEKQGQYHRDEGWKWGGCSADIRYGIGFAKVFVDAREIKQNARTLMNLHNNEAGRKILEENMKLECKCHGVSGSCTTKTCWTTLPQFRELGYVLKDKYNEAVHVEPVRASRNKRPTFLKIKKPLSYRKPMDTDLVYIEKSPNYC

SEQ ID NO: 76 - protein, 247 aa, artificial sequence
  human N-terminal domain (NTD) Wnt7a variant V68A
LGASIICNKIPGLAPRQRAICQSRPDAIIVIGEGSQMGLDECQFQFRNGRWNCSALGERTVFGKELKAGSREAAFTYAIIAAGVAHAITAACTQGNLSDCGCDKEKQGQYHRDEGWKWGGCSADIRYGIGFAKVFVDAREIKQNARTLMNLHNNEAGRKILEENMKLECKCHGVSGSCTTKTCWTTLPQFRELGYVLKDKYNEAVHVEPVRASRNKRPTFLKIKKPLSYRKPMDTDLVYIEKSPNYC

SEQ ID NO: 77 - protein, 247 aa, artificial sequence
  human N-terminal domain (NTD) Wnt7a variant F135A
LGASIICNKIPGLAPRQRAICQSRPDAIIVIGEGSQMGLDECQFQFRNGRWNCSALGERTVFGKELKVGSREAAFTYAIIAAGVAHAITAACTQGNLSDCGCDKEKQGQYHRDEGWKWGGCSADIRYGIGFAKVAVDAREIKQNARTLMNLHNNEAGRKILEENMKLECKCHGVSGSCTTKTCWTTLPQFRELGYVLKDKYNEAVHVEPVRASRNKRPTFLKIKKPLSYRKPMDTDLVYIEKSPNYC

SEQ ID NO: 78 - protein, 247 aa, artificial sequence
  human N-terminal domain (NTD) Wnt7a variant R146A
LGASIICNKIPGLAPRQRAICQSRPDAIIVIGEGSQMGLDECQFQFRNGRWNCSALGERTVFGKELKVGSREAAFTYAIIAAGVAHAITAACTQGNLSDCGCDKEKQGQYHRDEGWKWGGCSADIRYGIGFAKVFVDAREIKQNAATLMNLHNNEAGRKILEENMKLECKCHGVSGSCTTKTCWTTLPQFRELGYVLKDKYNEAVHVEPVRASRNKRPTFLKIKKPLSYRKPMDTDLVYIEKSPNYC

SEQ ID NO: 79 - protein, 247 aa, artificial sequence
  human N-terminal domain (NTD) Wnt7a variant K159S
LGASIICNKIPGLAPRQRAICQSRPDAIIVIGEGSQMGLDECQFQFRNGRWNCSALGERTVFGKELKVGSREAAFTYAIIAAGVAHAITAACTQGNLSDCGCDKEKQGQYHRDEGWKWGGCSADIRYGIGFAKVFVDAREIKQNARTLMNLHNNEAGRSILEENMKLECKCHGVSGSCTTKTCWTTLPQFRELGYVLKDKYNEAVHVEPVRASRNKRPTFLKIKKPLSYRKPMDTDLVYIEKSPNYC

SEQ ID NO: 80 - protein, 247 aa, artificial sequence
  human N-terminal domain (NTD) Wnt7a variant K159L
LGASIICNKIPGLAPRQRAICQSRPDAIIVIGEGSQMGLDECQFQFRNGRWNCSALGERTVFGKELKVGSREAAFTYAIIAAGVAHAITAACTQGNLSDCGCDKEKQGQYHRDEGWKWGGCSADIRYGIGFAKVFVDAREIKQNARTLMNLHNNEAGRLILEENMKLECKCHGVSGSCTTKTCWTTLPQFRELGYVLKDKYNEAVHVEPVRASRNKRPTFLKIKKPLSYRKPMDTDLVYIEKSPNYC

SEQ ID NO: 81 - protein, 247 aa, artificial sequence
  human N-terminal domain (NTD) Wnt7a variant K200A
LGASIICNKIPGLAPRQRAICQSRPDAIIVIGEGSQMGLDECQFQFRNGRWNCSALGERTVFGKELKVGSREAAFTYAIIAAGVAHAITAACTQGNLSDCGCDKEKQGQYHRDEGWKWGGCSADIRYGIGFAKVFVDAREIKQNARTLMNLHNNEAGRKILEENMKLECKCHGVSGSCTTKTCWTTLPQFRELGYVLKDAYNEAVHVEPVRASRNKRPTFLKIKKPLSYRKPMDTDLVYIEKSPNYC

SEQ ID NO: 82 - protein, 247 aa, artificial sequence
  human N-terminal domain (NTD) Wnt7a variant R214A
LGASIICNKIPGLAPRQRAICQSRPDAIIVIGEGSQMGLDECQFQFRNGRWNCSALGERTVFGKELKVGSREAAFTYAIIAAGVAHAITAACTQGNLSDCGCDKEKQGQYHRDEGWKWGGCSADIRYGIGFAKVFVDAREIKQNARTLMNLHNNEAGRKILEENMKLECKCHGVSGSCTTKTCWTTLPQFRELGYVLKDKYNEAVHVEPVRASANKRPTFLKIKKPLSYRKPMDTDLVYIEKSPNYC

SEQ ID NO: 83 - protein, 247 aa, artificial sequence; identical to SEQ ID NO: 24
  human N-terminal domain (NTD) Wnt7a variant P218A

SEQ ID NO: 84 - protein, 318 aa, artificial sequence
  human Wnt7a variant K318A
LGASIICNKIPGLAPRQRAICQSRPDAIIVIGEGSQMGLDECQFQFRNGRWNCSALGERTVFGKELKVGSREAAFTYAIIAAGVAHAITAACTQGNLSDCGCDKEKQGQYHRDEGWKWGGCSADIRYGIGFAKVFVDAREIKQNARTLMNLHNNEAGRKILEENMKLECKCHGVSGSCTTKTCWTTLPQFRELGYVLKDKYNEAVHVEPVRASRNKRPTFLKIKKPLSYRKPMDTDLVYIEKSPNYCEEDPVTGSVGTQGRACNKTAPQASGCDLMCCGRGYNTHQYARVWQCNCKFHWCCYVKCNTCSERTEMYTCA

SEQ ID NO: 85 - protein, 318 aa, artificial sequence
  human Wnt7a variant K159A
LGASIICNKIPGLAPRQRAICQSRPDAIIVIGEGSQMGLDECQFQFRNGRWNCSALGERTVFGKELKVGSREAAFTYAIIAAGVAHAITAACTQGNLSDCGCDKEKQGQYHRDEGWKWGGCSADIRYGIGFAKVFVDAREIKQNARTLMNLHNNEAGRAILEENMKLECKCHGVSGSCTTKTCWTTLPQFRELGYVLKDKYNEAVHVEPVRASRNKRPTFLKIKKPLSYRKPMDTDLVYIEKSPNYCEEDPVTGSVGTQGRACNKTAPQASGCDLMCCGRGYNTHQYARVWQCNCKFHWCCYVKCNTCSERTEMYTCK

SEQ ID NO: 86 - protein, 318 aa, artificial sequence
  human Wnt7a variant A27R
LGASIICNKIPGLAPRQRAICQSRPDRIIVIGEGSQMGLDECQFQFRNGRWNCSALGERTVFGKELKVGSREAAFTYAIIAAGVAHAITAACTQGNLSDCGCDKEKQGQYHRDEGWKWGGCSADIRYGIGFAKVFVDAREIKQNARTLMNLHNNEAGRKILEENMKLECKCHGVSGSCTTKTCWTTLPQFRELGYVLKDKYNEAVHVEPVRASRNKRPTFLKIKKPLSYRKPMDTDLVYIEKSPNYCEEDPVTGSVGTQGRACNKTAPQASGCDLMCCGRGYNTHQYARVWQCNCKFHWCCYVKCNTCSERTEMYTCK

SEQ ID NO: 87 - protein, 318 aa, artificial sequence
  human Wnt7a variant E33A
LGASIICNKIPGLAPRQRAICQSRPDAIIVIGAGSQMGLDECQFQFRNGRWNCSALGERTVFGKELKVGSREAAFTYAIIAAGVAHAITAACTQGNLSDCGCDKEKQGQYHRDEGWKWGGCSADIRYGIGFAKVFVDAREIKQNARTLMNLHNNEAGRKILEENMKLECKCHGVSGSCTTKTCWTTLPQFRELGYVLKDKYNEAVHVEPVRASRNKRPTFLKIKKPLSYRKPMDTDLVYIEKSPNYCEEDPVTGSVGTQGRACNKTAPQASGCDLMCCGRGYNTHQYARVWQCNCKFHWCCYVKCNTCSERTEMYTCK

SEQ ID NO: 88 - protein, 318 aa, artificial sequence
  human Wnt7a variant E41A
LGASIICNKIPGLAPRQRAICQSRPDAIIVIGEGSQMGLDACQFQFRNGRWNCSALGERTVFGKELKVGSREAAFTYAIIAAGVAHAITAACTQGNLSDCGCDKEKQGQYHRDEGWKWGGCSADIRYGIGFAKVFVDAREIKQNARTLMNLHNNEAGRKILEENMKLECKCHGVSGSCTTKTCWTTLPQFRELGYVLKDKYNEAVHVEPVRASRNKRPTFLKIKKPLSYRKPMDTDLVYIEKSPNYCEEDPVTGSVGTQGRACNKTAPQASGCDLMCCGRGYNTHQYARVWQCNCKFHWCCYVKCNTCSERTEMYTCK

SEQ ID NO: 89 - protein, 318 aa, artificial sequence
  human Wnt7a variant F44A
LGASIICNKIPGLAPRQRAICQSRPDAIIVIGEGSQMGLDECQAQFRNGRWNCSALGERTVFGKELKVGSREAAFTYAIIAAGVAHAITAACTQGNLSDCGCDKEKQGQYHRDEGWKWGGCSADIRYGIGFAKVFVDAREIKQNARTLMNLHNNEAGRKILEENMKLECKCHGVSGSCTTKTCWTTLPQFRELGYVLKDKYNEAVHVEPVRASRNKRPTFLKIKKPLSYRKPMDTDLVYIEKSPNYCEEDPVTGSVGTQGRACNKTAPQASGCDLMCCGRGYNTHQYARVWQCNCKFHWCCYVKCNTCSERTEMYTCK

SEQ ID NO: 90 - protein, 318 aa, artificial sequence
  human Wnt7a variant N52Q
LGASIICNKIPGLAPRQRAICQSRPDAIIVIGEGSQMGLDECQFQFRNGRWQCSALGERTVFGKELKVGSREAAFTYAIIAAGVAHAITAACTQGNLSDCGCDKEKQGQYHRDEGWKWGGCSADIRYGIGFAKVFVDAREIKQNARTLMNLHNNEAGRKILEENMKLECKCHGVSGSCTTKTCWTTLPQFRELGYVLKDKYNEAVHVEPVRASRNKRPTFLKIKKPLSYRKPMDTDLVYIEKSPNYCEEDPVTGSVGTQGRACNKTAPQASGCDLMCCGRGYNTHQYARVWQCNCKFHWCCYVKCNTCSERTEMYTCK

SEQ ID NO: 91 - protein, 318 aa, artificial sequence
  human Wnt7a variant I129A
LGASIICNKIPGLAPRQRAICQSRPDAIIVIGEGSQMGLDECQFQFRNGRWNCSALGERTVFGKELKVGSREAAFTYAIIAAGVAHAITAACTQGNLSDCGCDKEKQGQYHRDEGWKWGGCSADIRYGAGFAKVFVDAREIKQNARTLMNLHNNEAGRKILEENMKLECKCHGVSGSCTTKTCWTTLPQFRELGYVLKDKYNEAVHVEPVRASRNKRPTFLKIKKPLSYRKPMDTDLVYIEKSPNYCEEDPVTGSVGTQGRACNKTAPQASGCDLMCCGRGYNTHQYARVWQCNCKFHWCCYVKCNTCSERTEMYTCK

SEQ ID NO: 92 - protein, 318 aa, artificial sequence
  human Wnt7a variant F131A
LGASIICNKIPGLAPRQRAICQSRPDAIIVIGEGSQMGLDECQFQFRNGRWNCSALGERTVFGKELKVGSREAAFTYAIIAAGVAHAITAACTQGNLSDCGCDKEKQGQYHRDEGWKWGGCSADIRYGIGAAKVFVDAREIKQNARTLMNLHNNEAGRKILEENMKLECKCHGVSGSCTTKTCWTTLPQFRELGYVLKDKYNEAVHVEPVRASRNKRPTFLKIKKPLSYRKPMDTDLVYIEKSPNYCEEDPVTGSVGTQGRACNKTAPQASGCDLMCCGRGYNTHQYARVWQCNCKFHWCCYVKCNTCSERTEMYTCK

SEQ ID NO: 93 - protein, 318 aa, artificial sequence
  human Wnt7a variant K133A
LGASIICNKIPGLAPRQRAICQSRPDAIIVIGEGSQMGLDECQFQFRNGRWNCSALGERTVFGKELKVGSREAAFTYAIIAAGVAHAITAACTQGNLSDCGCDKEKQGQYHRDEGWKWGGCSADIRYGIGFAAVFVDAREIKQNARTLMNLHNNEAGRKILEENMKLECKCHGVSGSCTTKTCWTTLPQFRELGYVLKDKYNEAVHVEPVRASRNKRPTFLKIKKPLSYRKPMDTDLVYIEKSPNYCEEDPVTGSVGTQGRACNKTAPQASGCDLMCCGRGYNTHQYARVWQCNCKFHWCCYVKCNTCSERTEMYTCK

SEQ ID NO: 94 - protein, 318 aa, artificial sequence
  human Wnt7a variant I141A
LGASIICNKIPGLAPRQRAICQSRPDAIIVIGEGSQMGLDECQFQFRNGRWNCSALGERTVFGKELKVGSREAAFTYAIIAAGVAHAITAACTQGNLSDCGCDKEKQGQYHRDEGWKWGGCSADIRYGIGFAKVFVDAREAKQNARTLMNLHNNEAGRKILEENMKLECKCHGVSGSCTTKTCWTTLPQFRELGYVLKDKYNEAVHVEPVRASRNKRPTFLKIKKPLSYRKPMDTDLVYIEKSPNYCEEDPVTGSVGTQGRACNKTAPQASGCDLMCCGRGYNTHQYARVWQCNCKFHWCCYVKCNTCSERTEMYTCK

SEQ ID NO: 95 - protein, 318 aa, artificial sequence
  human Wnt7a variant R158A
LGASIICNKIPGLAPRQRAICQSRPDAIIVIGEGSQMGLDECQFQFRNGRWNCSALGERTVFGKELKVGSREAAFTYAIIAAGVAHAITAACTQGNLSDCGCDKEKQGQYHRDEGWKWGGCSADIRYGIGFAKVFVDAREIKQNARTLMNLHNNEAGAKILEENMKLECKCHGVSGSCTTKTCWTTLPQFRELGYVLKDKYNEAVHVEPVRASRNKRPTFLKIKKPLSYRKPMDTDLVYIEKSPNYCEEDPVTGSVGTQGRACNKTAPQASGCDLMCCGRGYNTHQYARVWQCNCKFHWCCYVKCNTCSERTEMYTCK

SEQ ID NO: 96 - protein, 318 aa, artificial sequence
  human Wnt7a variant K181A
LGASIICNKIPGLAPRQRAICQSRPDAIIVIGEGSQMGLDECQFQFRNGRWNCSALGERTVFGKELKVGSREAAFTYAIIAAGVAHAITAACTQGNLSDCGCDKEKQGQYHRDEGWKWGGCSADIRYGIGFAKVFVDAREIKQNARTLMNLHNNEAGRKILEENMKLECKCHGVSGSCTTATCWTTLPQFRELGYVLKDKYNEAVHVEPVRASRNKRPTFLKIKKPLSYRKPMDTDLVYIEKSPNYCEEDPVTGSVGTQGRACNKTAPQASGCDLMCCGRGYNTHQYARVWQCNCKFHWCCYVKCNTCSERTEMYTCK

SEQ ID NO: 97 - protein, 318 aa, artificial sequence
  human Wnt7a variant R191A
LGASIICNKIPGLAPRQRAICQSRPDAIIVIGEGSQMGLDECQFQFRNGRWNCSALGERTVFGKELKVGSREAAFTYAIIAAGVAHAITAACTQGNLSDCGCDKEKQGQYHRDEGWKWGGCSADIRYGIGFAKVFVDAREIKQNARTLMNLHNNEAGRKILEENMKLECKCHGVSGSCTTKTCWTTLPQFAELGYVLKDKYNEAVHVEPVRASRNKRPTFLKIKKPLSYRKPMDTDLVYIEKSPNYCEEDPVTGSVGTQGRACNKTAPQASGCDLMCCGRGYNTHQYARVWQCNCKFHWCCYVKCNTCSERTEMYTCK

SEQ ID NO: 98 - protein, 318 aa, artificial sequence
  human Wnt7a variant K198A
LGASIICNKIPGLAPRQRAICQSRPDAIIVIGEGSQMGLDECQFQFRNGRWNCSALGERTVFGKELKVGSREAAFTYAIIAAGVAHAITAACTQGNLSDCGCDKEKQGQYHRDEGWKWGGCSADIRYGIGFAKVFVDAREIKQNARTLMNLHNNEAGRKILEENMKLECKCHGVSGSCTTKTCWTTLPQFRELGYVLADKYNEAVHVEPVRASRNKRPTFLKIKKPLSYRKPMDTDLVYIEKSPNYCEEDPVTGSVGTQGRACNKTAPQASGCDLMCCGRGYNTHQYARVWQCNCKFHWCCYVKCNTCSERTEMYTCK

SEQ ID NO: 99 - protein, 317 aa, artificial sequence
  human Wnt7a variant V205A
LGASIICNKIPGLAPRQRAICQSRPDAIIVIGEGSQMGLDECQFQFRNGRWNCSALGERTVFGKELKVGSREAAFTYAIIAAGVAHAITAACTQGNLSDCGCDKEKQGQYHRDEGWKWGGCSADIRYGIGFAKVFVDAREIKQNARTLMNLHNNEAGRKILEENMKLECKCHGVSGSCTTKTCWTTLPQFRELGYVLKDKYNEAAHVEPVRASRNKRPTFLKIKKPLSYRKPMDTDLVYIEKSPNYEEDPVTGSVGTQGRACNKTAPQASGCDLMCCGRGYNTHQYARVWQCNCKFHWCCYVKCNTCSERTEMYTCK

SEQ ID NO: 100 - protein, 318 aa, artificial sequence
  human Wnt7a variant E208A
LGASIICNKIPGLAPRQRAICQSRPDAIIVIGEGSQMGLDECQFQFRNGRWNCSALGERTVFGKELKVGSREAAFTYAIIAAGVAHAITAACTQGNLSDCGCDKEKQGQYHRDEGWKWGGCSADIRYGIGFAKVFVDAREIKQNARTLMNLHNNEAGRKILEENMKLECKCHGVSGSCTTKTCWTTLPQFRELGYVLKDKYNEAVHVAPVRASRNKRPTFLKIKKPLSYRKPMDTDLVYIEKSPNYCEEDPVTGSVGTQGRACNKTAPQASGCDLMCCGRGYNTHQYARVWQCNCKFHWCCYVKCNTCSERTEMYTCK

SEQ ID NO: 101 - protein, 318 aa, artificial sequence
  human Wnt7a variant K216A
LGASIICNKIPGLAPRQRAICQSRPDAIIVIGEGSQMGLDECQFQFRNGRWNCSALGERTVFGKELKVGSREAAFTYAIIAAGVAHAITAACTQGNLSDCGCDKEKQGQYHRDEGWKWGGCSADIRYGIGFAKVFVDAREIKQNARTLMNLHNNEAGRKILEENMKLECKCHGVSGSCTTKTCWTTLPQFRELGYVLKDKYNEAVHVEPVRASRNARPTFLKIKKPLSYRKPMDTDLVYIEKSPNYCEEDPVTGSVGTQGRACNKTAPQASGCDLMCCGRGYNTHQYARVWQCNCKFHWCCYVKCNTCSERTEMYTCK

SEQ ID NO: 102 - protein, 318 aa, artificial sequence
  human Wnt7a variant K222A
LGASIICNKIPGLAPRQRAICQSRPDAIIVIGEGSQMGLDECQFQFRNGRWNCSALGERTVFGKELKVGSREAAFTYAIIAAGVAHAITAACTQGNLSDCGCDKEKQGQYHRDEGWKWGGCSADIRYGIGFAKVFVDAREIKQNARTLMNLHNNEAGRKILEENMKLECKCHGVSGSCTTKTCWTTLPQFRELGYVLKDKYNEAVHVEPVRASRNKRPTFLAIKKPLSYRKPMDTDLVYIEKSPNYCEEDPVTGSVGTQGRACNKTAPQASGCDLMCCGRGYNTHQYARVWQCNCKFHWCCYVKCNTCSERTEMYTCK

SEQ ID NO: 103 - protein, 318 aa, artificial sequence
  human Wnt7a variant I223A
LGASIICNKIPGLAPRQRAICQSRPDAIIVIGEGSQMGLDECQFQFRNGRWNCSALGERTVFGKELKVGSREAAFTYAIIAAGVAHAITAACTQGNLSDCGCDKEKQGQYHRDEGWKWGGCSADIRYGIGFAKVFVDAREIKQNARTLMNLHNNEAGRKILEENMKLECKCHGVSGSCTTKTCWTTLPQFRELGYVLKDKYNEAVHVEPVRASRNKRPTFLKAKKPLSYRKPMDTDLVYIEKSPNYCEEDPVTGSVGTQGRACNKTAPQASGCDLMCCGRGYNTHQYARVWQCNCKFHWCCYVKCNTCSERTEMYTCK

SEQ ID NO: 104 - protein, 318 aa, artificial sequence
  human Wnt7a variant Y229A
LGASIICNKIPGLAPRQRAICQSRPDAIIVIGEGSQMGLDECQFQFRNGRWNCSALGERTVFGKELKVGSREAAFTYAIIAAGVAHAITAACTQGNLSDCGCDKEKQGQYHRDEGWKWGGCSADIRYGIGFAKVFVDAREIKQNARTLMNLHNNEAGRKILEENMKLECKCHGVSGSCTTKTCWTTLPQFRELGYVLKDKYNEAVHVEPVRASRNKRPTFLKIKKPLSARKPMDTDLVYIEKSPNYCEEDPVTGSVGTQGRACNKTAPQASGCDLMCCGRGYNTHQYARVWQCNCKFHWCCYVKCNTCSERTEMYTCK

SEQ ID NO: 105 - protein, 318 aa, artificial sequence
  human Wnt7a variant P232A
LGASIICNKIPGLAPRQRAICQSRPDAIIVIGEGSQMGLDECQFQFRNGRWNCSALGERTVFGKELKVGSREAAFTYAIIAAGVAHAITAACTQGNLSDCGCDKEKQGQYHRDEGWKWGGCSADIRYGIGFAKVFVDAREIKQNARTLMNLHNNEAGRKILEENMKLECKCHGVSGSCTTKTCWTTLPQFRELGYVLKDKYNEAVHVEPVRASRNKRPTFLKIKKPLSYRKAMDTDLVYIEKSPNYCEEDPVTGSVGTQGRACNKTAPQASGCDLMCCGRGYNTHQYARVWQCNCKFHWCCYVKCNTCSERTEMYTCK

SEQ ID NO: 106 - protein, 318 aa, artificial sequence
  human Wnt7a variant T235A
LGASIICNKIPGLAPRQRAICQSRPDAIIVIGEGSQMGLDECQFQFRNGRWNCSALGERTVFGKELKVGSREAAFTYAIIAAGVAHAITAACTQGNLSDCGCDKEKQGQYHRDEGWKWGGCSADIRYGIGFAKVFVDAREIKQNARTLMNLHNNEAGRKILEENMKLECKCHGVSGSCTTKTCWTTLPQFRELGYVLKDKYNEAVHVEPVRASRNKRPTFLKIKKPLSYRKPMDADLVYIEKSPNYCEEDPVTGSVGTQGRACNKTAPQASGCDLMCCGRGYNTHQYARVWQCNCKFHWCCYVKCNTCSERTEMYTCK

SEQ ID NO: 107 - protein, 318 aa, artificial sequence
  human Wnt7a variant Q17A
LGASIICNKIPGLAPRARAICQSRPDAIIVIGEGSQMGLDECQFQFRNGRWNCSALGERTVFGKELKVGSREAAFTYAIIAAGVAHAITAACTQGNLSDCGCDKEKQGQYHRDEGWKWGGCSADIRYGIGFAKVFVDAREIKQNARTLMNLHNNEAGRKILEENMKLECKCHGVSGSCTTKTCWTTLPQFRELGYVLKDKYNEAVHVEPVRASRNKRPTFLKIKKPLSYRKPMDTDLVYIEKSPNYCEEDPVTGSVGTQGRACNKTAPQASGCDLMCCGRGYNTHQYARVWQCNCKFHWCCYVKCNTCSERTEMYTCK

SEQ ID NO: 108 - protein, 318 aa, artificial sequence
  human Wnt7a variant I20A
LGASIICNKIPGLAPRQRAACQSRPDAIIVIGEGSQMGLDECQFQFRNGRWNCSALGERTVFGKELKVGSREAAFTYAIIAAGVAHAITAACTQGNLSDCGCDKEKQGQYHRDEGWKWGGCSADIRYGIGFAKVFVDAREIKQNARTLMNLHNNEAGRKILEENMKLECKCHGVSGSCTTKTCWTTLPQFRELGYVLKDKYNEAVHVEPVRASRNKRPTFLKIKKPLSYRKPMDTDLVYIEKSPNYCEEDPVTGSVGTQGRACNKTAPQASGCDLMCCGRGYNTHQYARVWQCNCKFHWCCYVKCNTCSERTEMYTCK

SEQ ID NO: 109 - protein, 318 aa, artificial sequence
  human Wnt7a variant P25A
LGASIICNKIPGLAPRQRAICQSRADAIIVIGEGSQMGLDECQFQFRNGRWNCSALGERTVFGKELKVGSREAAFTYAIIAAGVAHAITAACTQGNLSDCGCDKEKQGQYHRDEGWKWGGCSADIRYGIGFAKVFVDAREIKQNARTLMNLHNNEAGRKILEENMKLECKCHGVSGSCTTKTCWTTLPQFRELGYVLKDKYNEAVHVEPVRASRNKRPTFLKIKKPLSYRKPMDTDLVYIEKSPNYCEEDPVTGSVGTQGRACNKTAPQASGCDLMCCGRGYNTHQYARVWQCNCKFHWCCYVKCNTCSERTEMYTCK

SEQ ID NO: 110 - protein, 318 aa, artificial sequence
  human Wnt7a variant M37A
LGASIICNKIPGLAPRQRAICQSRPDAIIVIGEGSQAGLDECQFQFRNGRWNCSALGERTVFGKELKVGSREAAFTYAIIAAGVAHAITAACTQGNLSDCGCDKEKQGQYHRDEGWKWGGCSADIRYGIGFAKVFVDAREIKQNARTLMNLHNNEAGRKILEENMKLECKCHGVSGSCTTKTCWTTLPQFRELGYVLKDKYNEAVHVEPVRASRNKRPTFLKIKKPLSYRKPMDTDLVYIEKSPNYCEEDPVTGSVGTQGRACNKTAPQASGCDLMCCGRGYNTHQYARVWQCNCKFHWCCYVKCNTCSERTEMYTCK

SEQ ID NO: 111 - protein, 318 aa, artificial sequence
  human Wnt7a variant L39A
LGASIICNKIPGLAPRQRAICQSRPDAIIVIGEGSQMGADECQFQFRNGRWNCSALGERTVFGKELKVGSREAAFTYAIIAAGVAHAITAACTQGNLSDCGCDKEKQGQYHRDEGWKWGGCSADIRYGIGFAKVFVDAREIKQNARTLMNLHNNEAGRKILEENMKLECKCHGVSGSCTTKTCWTTLPQFRELGYVLKDKYNEAVHVEPVRASRNKRPTFLKIKKPLSYRKPMDTDLVYIEKSPNYCEEDPVTGSVGTQGRACNKTAPQASGCDLMCCGRGYNTHQYARVWQCNCKFHWCCYVKCNTCSERTEMYTCK

SEQ ID NO: 112 - protein, 318 aa, artificial sequence
  human Wnt7a variant I28A
LGASIICNKIPGLAPRQRAICQSRPDAAIVIGEGSQMGLDECQFQFRNGRWNCSALGERTVFGKELKVGSREAAFTYAIIAAGVAHAITAACTQGNLSDCGCDKEKQGQYHRDEGWKWGGCSADIRYGIGFAKVFVDAREIKQNARTLMNLHNNEAGRKILEENMKLECKCHGVSGSCTTKTCWTTLPQFRELGYVLKDKYNEAVHVEPVRASRNKRPTFLKIKKPLSYRKPMDTDLVYIEKSPNYCEEDPVTGSVGTQGRACNKTAPQASGCDLMCCGRGYNTHQYARVWQCNCKFHWCCYVKCNTCSERTEMYTCK

SEQ ID NO: 113 - protein, 318 aa, artificial sequence
  human Wnt7a variant R50A
LGASIICNKIPGLAPRQRAICQSRPDAIIVIGEGSQMGLDECQFQFRNGAWNCSALGERTVFGKELKVGSREAAFTYAIIAAGVAHAITAACTQGNLSDCGCDKEKQGQYHRDEGWKWGGCSADIRYGIGFAKVFVDAREIKQNARTLMNLHNNEAGRKILEENMKLECKCHGVSGSCTTKTCWTTLPQFRELGYVLKDKYNEAVHVEPVRASRNKRPTFLKIKKPLSYRKPMDTDLVYIEKSPNYCEEDPVTGSVGTQGRACNKTAPQASGCDLMCCGRGYNTHQYARVWQCNCKFHWCCYVKCNTCSERTEMYTCK

SEQ ID NO: 114 - protein, 318 aa, artificial sequence
  human Wnt7a variant V68A
LGASIICNKIPGLAPRQRAICQSRPDAIIVIGEGSQMGLDECQFQFRNGRWNCSALGERTVFGKELKAGSREAAFTYAIIAAGVAHAITAACTQGNLSDCGCDKEKQGQYHRDEGWKWGGCSADIRYGIGFAKVFVDAREIKQNARTLMNLHNNEAGRKILEENMKLECKCHGVSGSCTTKTCWTTLPQFRELGYVLKDKYNEAVHVEPVRASRNKRPTFLKIKKPLSYRKPMDTDLVYIEKSPNYCEEDPVTGSVGTQGRACNKTAPQASGCDLMCCGRGYNTHQYARVWQCNCKFHWCCYVKCNTCSERTEMYTCK

SEQ ID NO: 115 - protein, 318 aa, artificial sequence
  human Wnt7a variant F135A
LGASIICNKIPGLAPRQRAICQSRPDAIIVIGEGSQMGLDECQFQFRNGRWNCSALGERTVFGKELKVGSREAAFTYAIIAAGVAHAITAACTQGNLSDCGCDKEKQGQYHRDEGWKWGGCSADIRYGIGFAKVAVDAREIKQNARTLMNLHNNEAGRKILEENMKLECKCHGVSGSCTTKTCWTTLPQFRELGYVLKDKYNEAVHVEPVRASRNKRPTFLKIKKPLSYRKPMDTDLVYIEKSPNYCEEDPVTGSVGTQGRACNKTAPQASGCDLMCCGRGYNTHQYARVWQCNCKFHWCCYVKCNTCSERTEMYTCK

SEQ ID NO: 116 - protein, 318 aa, artificial sequence
  human Wnt7a variant R146A
LGASIICNKIPGLAPRQRAICQSRPDAIIVIGEGSQMGLDECQFQFRNGRWNCSALGERTVFGKELKVGSREAAFTYAIIAAGVAHAITAACTQGNLSDCGCDKEKQGQYHRDEGWKWGGCSADIRYGIGFAKVFVDAREIKQNAATLMNLHNNEAGRKILEENMKLECKCHGVSGSCTTKTCWTTLPQFRELGYVLKDKYNEAVHVEPVRASRNKRPTFLKIKKPLSYRKPMDTDLVYIEKSPNYCEEDPVTGSVGTQGRACNKTAPQASGCDLMCCGRGYNTHQYARVWQCNCKFHWCCYVKCNTCSERTEMYTCK

SEQ ID NO: 117 - protein, 318 aa, artificial sequence
  human Wnt7a variant K159S
LGASIICNKIPGLAPRQRAICQSRPDAIIVIGEGSQMGLDECQFQFRNGRWNCSALGERTVFGKELKVGSREAAFTYAIIAAGVAHAITAACTQGNLSDCGCDKEKQGQYHRDEGWKWGGCSADIRYGIGFAKVFVDAREIKQNARTLMNLHNNEAGRSILEENMKLECKCHGVSGSCTTKTCWTTLPQFRELGYVLKDKYNEAVHVEPVRASRNKRPTFLKIKKPLSYRKPMDTDLVYIEKSPNYCEEDPVTGSVGTQGRACNKTAPQASGCDLMCCGRGYNTHQYARVWQCNCKFHWCCYVKCNTCSERTEMYTCK

SEQ ID NO: 118 - protein, 318 aa, artificial sequence
  human Wnt7a variant K159L
LGASIICNKIPGLAPRQRAICQSRPDAIIVIGEGSQMGLDECQFQFRNGRWNCSALGERTVFGKELKVGSREAAFTYAIIAAGVAHAITAACTQGNLSDCGCDKEKQGQYHRDEGWKWGGCSADIRYGIGFAKVFVDAREIKQNARTLMNLHNNEAGRLILEENMKLECKCHGVSGSCTTKTCWTTLPQFRELGYVLKDKYNEAVHVEPVRASRNKRPTFLKIKKPLSYRKPMDTDLVYIEKSPNYCEEDPVTGSVGTQGRACNKTAPQASGCDLMCCGRGYNTHQYARVWQCNCKFHWCCYVKCNTCSERTEMYTCK

SEQ ID NO: 119 - protein, 318 aa, artificial sequence
  human Wnt7a variant K200A
LGASIICNKIPGLAPRQRAICQSRPDAIIVIGEGSQMGLDECQFQFRNGRWNCSALGERTVFGKELKVGSREAAFTYAIIAAGVAHAITAACTQGNLSDCGCDKEKQGQYHRDEGWKWGGCSADIRYGIGFAKVFVDAREIKQNARTLMNLHNNEAGRKILEENMKLECKCHGVSGSCTTKTCWTTLPQFRELGYVLKDAYNEAVHVEPVRASRNKRPTFLKIKKPLSYRKPMDTDLVYIEKSPNYCEEDPVTGSVGTQGRACNKTAPQASGCDLMCCGRGYNTHQYARVWQCNCKFHWCCYVKCNTCSERTEMYTCK

SEQ ID NO: 120 - protein, 318 aa, artificial sequence
  human Wnt7a variant R214A
LGASIICNKIPGLAPRQRAICQSRPDAIIVIGEGSQMGLDECQFQFRNGRWNCSALGERTVFGKELKVGSREAAFTYAIIAAGVAHAITAACTQGNLSDCGCDKEKQGQYHRDEGWKWGGCSADIRYGIGFAKVFVDAREIKQNARTLMNLHNNEAGRKILEENMKLECKCHGVSGSCTTKTCWTTLPQFRELGYVLKDKYNEAVHVEPVRASANKRPTFLKIKKPLSYRKPMDTDLVYIEKSPNYCEEDPVTGSVGTQGRACNKTAPQASGCDLMCCGRGYNTHQYARVWQCNCKFHWCCYVKCNTCSERTEMYTCK

SEQ ID NO: 121 - protein, 318 aa, artificial sequence; identical to SEQ ID NO: 51
  human Wnt7a variant P218A